European Patent Specification EP 4 281 484 B1, published March 18, 2026. Title: ANTI-HER-2/TROP-2 CONSTRUCTS AND USES THEREOF. Applicant: BiOneCure Therapeutics, Inc. Application Not Yet Assigned. The sequence listing filed with the application follows.

SEQUENCE LISTING (63 sequences)

SEQ ID NO: 1 - protein, 1225 aa, Artificial Sequence
  Synthetic Construct
MKLRLPASPETHLDMLRHLYQGCQVVQGNLELTYLPTNASLSFLQDIQEVQGYVLIAHNQVRQVPLQRLRIVRGTQLFEDNYALAVLDNGDPLNNTTPVTGASPGGLRELQLRSLTEILKGGVLIQRNPQLCYQDTILWKDIFHKNNQLALTLIDTNRSRACHPCSPMCKGSRCWGESSEDCQSLTRTVCAGGCARCKGPLPTDCCHEQCAAGCTGPKHSDCLACLHFNHSGICELHCPALVTYNTDTFESMPNPEGRYTFGASCVTACPYNYLSTDVGSCTLVCPLHNQEVTAEDGTQRCEKCSKPCARVCYGLGMEHLREVRAVTSANIQEFAGCKKIFGSLAFLPESFDGDPASNTAPLQPEQLQVFETLEEITGYLYISAWPDSLPDLSVFQNLQVIRGRILHNGAYSLTLQGLGISWLGLRSLRELGSGLALIHHNTHLCFVHTVPWDQLFRNPHQALLHTANRPEDECVGEGLACHQLCARGHCWGPGPTQCVNCSQFLRGQECVEECRVLQGLPREYVNARHCLPCHPECQPQNGSVTCFGPEADQCVACAHYKDPPFCVARCPSGVKPDLSYMPIWKFPDEEGACQPCPINCTHSCVDLDDKGCPAEQRASPLTSIISAVVGILLVVVLGVVFGILIKRRQQKIRKYTMRRLLQETELVEPLTPSGAMPNQAQMRILKETELRKVKVLGSGAFGTVYKGIWIPDGENVKIPVAIKVLRENTSPKANKEILDEAYVMAGVGSPYVSRLLGICLTSTVQLVTQLMPYGCLLDHVRENRGRLGSQDLLNWCMQIAKGMSYLEDVRLVHRDLAARNVLVKSPNHVKITDFGLARLLDIDETEYHADGGKVPIKWMALESILRRRFTHQSDVWSYGVTVWELMTFGAKPYDGIPAREIPDLLEKGERLPQPPICTIDVYMIMVKCWMIDSECRPRFRELVSEFSRMARDPQRFVVIQNEDLGPASPLDSTFYRSLLEDDDMGDLVDAEEYLVPQQGFFCPDPAPGAGGMVHHRHRSSSTRSGGGDLTLGLEPSEEEAPRSPLAPSEGAGSDVFDGDLGMGAAKGLQSLPTHDPSPLQRYSEDPTVPLPSETDGYVAPLTCSPQPEYVNQPDVRPQPPSPREGPLPAARPAGATLERPKTLSPGKNGVVKDVFAFGGAVENPEYLTPQGGAAPQPHPPPAFSPAFDNLYYWDQDPPERGAPPSTFKGTPTAENPEYLGLDVPV

SEQ ID NO: 2 - protein, 322 aa, Artificial Sequence
  Synthetic Construct
MARGPGLAPPPLRLPLLLLVLAAVTGHTAAQDNCTCPTNKMTVCSPDGPGGRCQCALGSGMAVDCSTLTSKCLLLKARMSAPKNARTLVRPSEHALVDNDGLYDPDCDPEGRFKARQCNQTSVCWCVNSVGVRRTDKGDLSLRCDELVRTHHILIDLRHRPTAGAFNHSDLDAELRRLFRERYRLHPKFVAAVHYEQPTIQIELRQNTSQKAAGDVDIGDAAYYFERDIKGESLFQGRGGLDLRVRGEPLQVERTLIYYLDEIPPKFSMKRLTAGLIAVIVVVVVALVAGMAVLVITNRRKSGKYKKVEIKELGELRKEPSL

SEQ ID NO: 3 - protein, 242 aa, Artificial Sequence
  Synthetic Construct
DIQMTQSPSSLSASVGDRVTITCRASQDVNTAVAWYQQKPGKAPKLLIYSASFLYSGVPSRFSGSRSGTDFTLTISSLQPEDFATYYCQQHYTTPPTFGQGTKVEIKGGGGSGGGGSGGGGSEVQLVESGGGLVQPGGSLRLSCAASGFNIKDTYIHWVRQAPGKGLEWVARIYPTNGYTRYADSVKGRFTISADTSKNTAYLQMNSLRAEDTAVYYCSRWGGDGFYAMDYWGQGTLVTVSS

SEQ ID NO: 4 - protein, 119 aa, Artificial Sequence
  Synthetic Construct
QVQLQESGPGLVKPSETLSLTCTVSGFSLTSYGVNWIRQPPGKGLEWIGVMWAGGSTNYNSALMSRLTISKDTSKNQFSLKLSSVTAADTAVYYCARDENWDGAWFAYWGQGTLVTVSS

SEQ ID NO: 5 - protein, 112 aa, Artificial Sequence
  Synthetic Construct
DIVMTQSPDSLAVSLGERATINCKSSQSLLNSGTRKNYLAWYQQKPGQPPKLLISWASSRESGVPDRFSGSGSGTDFTLTISSLQAEDVAVYYCKQSYNLFTFGGGTKVEIK

SEQ ID NO: 6 - protein, 246 aa, Artificial Sequence
  Synthetic Construct
DIVMTQSPDSLAVSLGERATINCKSSQSLLNSGTRKNYLAWYQQKPGQPPKLLISWASSRESGVPDRFSGSGSGTDFTLTISSLQAEDVAVYYCKQSYNLFTFGGGTKVEIKGGGGSGGGGSGGGGSQVQLQESGPGLVKPSETLSLTCTVSGFSLTSYGVNWIRQPPGKGLEWIGVMWAGGSTNYNSALMSRLTISKDTSKNQFSLKLSSVTAADTAVYYCARDENWDGAWFAYWGQGTLVTVSS

SEQ ID NO: 7 - protein, 120 aa, Artificial Sequence [sequence omitted]

SEQ ID NO: 8 - protein, 107 aa, Artificial Sequence [sequence omitted]

SEQ ID NO: 9 - protein, 243 aa, Artificial Sequence
  Synthetic Construct
DIQLTQSPSSLSASVGDRVSITCKASQDVSIAVAWYQQKPGKAPKLLIYSASYRYTGVPDRFSGSGSGTDFTLTISSLQPEDFAVYYCQQHYITPLTFGAGTKVDIKGGGGSGGGGSGGGGSQVQLQQSGSELKKPGASVKVSCKASGYTFTNYGMNWVKQAPGQGLKWMGWINTYTGEPTYTDDFKGRFAFSLDTSVSTAYLQISSLKADDTAVYFCARGGFGSSYWYFDVWGQGSLVTVSS

SEQ ID NO: 10 - protein, 121 aa, Artificial Sequence
  Synthetic Construct
QVQLQQSGSELKKPGASVKVSCKASGYTFTNYGMNWVKQAPGQGLKWMGWINTYTGEPTYTDDFKGRFAFSLDTSVSTAYLQISSLKADDTAVYFCARGGFGSSYWYFDVWGQGSLVTVSS

SEQ ID NO: 11 - protein, 107 aa, Artificial Sequence
  Synthetic Construct
DIQLTQSPSSLSASVGDRVSITCKASQDVSIAVAWYQQKPGKAPKLLIYSASYRYTGVPDRFSGSGSGTDFTLTISSLQPEDFAVYYCQQHYITPLTFGAGTKVDIK

SEQ ID NO: 12 - protein, 330 aa, Artificial Sequence
  Synthetic Construct
ASTKGPSVFPLAPSSKSTSGGTAALGCLVKDYFPEPVTVSWNSGALTSGVHTFPAVLQSSGLYSLSSVVTVPSSSLGTQTYICNVNHKPSNTKVDKRVEPKSCDKTHTCPPCPAPELLGGPSVFLFPPKPKDTLMISRTPEVTCVVVDVSHEDPEVKFNWYVDGVEVHNAKTKPREEQYNSTYRVVSVLTVLHQDWLNGKEYKCKVSNKALPAPIEKTISKAKGQPREPQVYTLPPSREEMTKNQVSLTCLVKGFYPSDIAVEWESNGQPENNYKTTPPVLDSDGSFFLYSKLTVDKSRWQQGNVFSCSVMHEALHNHYTQKSLSLSPGK

SEQ ID NO: 13 - protein, 107 aa, Artificial Sequence [sequence omitted]

SEQ ID NO: 14 - protein, 705 aa, Artificial Sequence
  Synthetic Construct
DIQMTQSPSSLSASVGDRVTITCRASQDVNTAVAWYQQKPGKAPKLLIYSASFLYSGVPSRFSGSRSGTDFTLTISSLQPEDFATYYCQQHYTTPPTFGQGTKVEIKGGGGSGGGGSGGGGSEVQLVESGGGLVQPGGSLRLSCAASGFNIKDTYIHWVRQAPGKGLEWVARIYPTNGYTRYADSVKGRFTISADTSKNTAYLQMNSLRAEDTAVYYCSRWGGDGFYAMDYWGQGTLVTVSSGGGGSGGGGSGGGSQVQLQESGPGLVKPSETLSLTCTVSGFSLTSYGVNWIRQPPGKGLEWIGVMWAGGSTNYNSALMSRLTISKDTSKNQFSLKLSSVTAADTAVYYCARDENWDGAWFAYWGQGTLVTVSSASTKGPSVFPLAPSSKSTSGGTAALGCLVKDYFPEPVTVSWNSGALTSGVHTFPAVLQSSGLYSLSSVVTVPSSSLGTQTYICNVNHKPSNTKVDKRVEPKSCDKTHTCPPCPAPELLGGPSVFLFPPKPKDTLMISRTPEVTCVVVDVSHEDPEVKFNWYVDGVEVHNAKTKPREEQYNSTYRVVSVLTVLHQDWLNGKEYKCKVSNKALPAPIEKTISKAKGQPREPQVYTLPPSREEMTKNQVSLTCLVKGFYPSDIAVEWESNGQPENNYKTTPPVLDSDGSFFLYSKLTVDKSRWQQGNVFSCSVMHEALHNHYTQKSLSLSPGK

SEQ ID NO: 15 - protein, 219 aa, Artificial Sequence
  Synthetic Construct
DIVMTQSPDSLAVSLGERATINCKSSQSLLNSGTRKNYLAWYQQKPGQPPKLLISWASSRESGVPDRFSGSGSGTDFTLTISSLQAEDVAVYYCKQSYNLFTFGGGTKVEIKRTVAAPSVFIFPPSDEQLKSGTASVVCLLNNFYPREAKVQWKVDNALQSGNSQESVTEQDSKDSTYSLSSTLTLSKADYEKHKVYACEVTHQGLSSPVTKSFNRGEC

SEQ ID NO: 16 - protein, 710 aa, Artificial Sequence
  Synthetic Construct
DIVMTQSPDSLAVSLGERATINCKSSQSLLNSGTRKNYLAWYQQKPGQPPKLLISWASSRESGVPDRFSGSGSGTDFTLTISSLQAEDVAVYYCKQSYNLFTFGGGTKVEIKGGGGSGGGGSGGGGSQVQLQESGPGLVKPSETLSLTCTVSGFSLTSYGVNWIRQPPGKGLEWIGVMWAGGSTNYNSALMSRLTISKDTSKNQFSLKLSSVTAADTAVYYCARDENWDGAWFAYWGQGTLVTVSSGGGGSGGGGSGGGSEVQLVESGGGLVQPGGSLRLSCAASGFNIKDTYIHWVRQAPGKGLEWVARIYPTNGYTRYADSVKGRFTISADTSKNTAYLQMNSLRAEDTAVYYCSRWGGDGFYAMDYWGQGTLVTVSSASTKGPSVFPLAPSSKSTSGGTAALGCLVKDYFPEPVTVSWNSGALTSGVHTFPAVLQSSGLYSLSSVVTVPSSSLGTQTYICNVNHKPSNTKVDKRVEPKSCDKTHTCPPCPAPELLGGPSVFLFPPKPKDTLMISRTPEVTCVVVDVSHEDPEVKFNWYVDGVEVHNAKTKPREEQYNSTYRVVSVLTVLHQDWLNGKEYKCKVSNKALPAPIEKTISKAKGQPREPQVYTLPPSREEMTKNQVSLTCLVKGFYPSDIAVEWESNGQPENNYKTTPPVLDSDGSFFLYSKLTVDKSRWQQGNVFSCSVMHEALHNHYTQKSLSLSPGK

SEQ ID NO: 17 - protein, 214 aa, Artificial Sequence
  Synthetic Construct
DIQMTQSPSSLSASVGDRVTITCRASQDVNTAVAWYQQKPGKAPKLLIYSASFLYSGVPSRFSGSRSGTDFTLTISSLQPEDFATYYCQQHYTTPPTFGQGTKVEIKRTVAAPSVFIFPPSDEQLKSGTASVVCLLNNFYPREAKVQWKVDNALQSGNSQESVTEQDSKDSTYSLSSTLTLSKADYEKHKVYACEVTHQGLSSPVTKSFNRGEC

SEQ ID NO: 18 - protein, 702 aa, Artificial Sequence
  Synthetic Construct
EVQLVESGGGLVQPGGSLRLSCAASGFNIKDTYIHWVRQAPGKGLEWVARIYPTNGYTRYADSVKGRFTISADTSKNTAYLQMNSLRAEDTAVYYCSRWGGDGFYAMDYWGQGTLVTVSSASTKGPSVFPLAPSSKSTSGGTAALGCLVKDYFPEPVTVSWNSGALTSGVHTFPAVLQSSGLYSLSSVVTVPSSSLGTQTYICNVNHKPSNTKVDKRVEPKSCDKTHTCPPCPAPELLGGPSVFLFPPKPKDTLMISRTPEVTCVVVDVSHEDPEVKFNWYVDGVEVHNAKTKPREEQYNSTYRVVSVLTVLHQDWLNGKEYKCKVSNKALPAPIEKTISKAKGQPREPQVYTLPPSREEMTKNQVSLTCLVKGFYPSDIAVEWESNGQPENNYKTTPPVLDSDGSFFLYSKLTVDKSRWQQGNVFSCSVMHEALHNHYTQKSLSLSPGGGGGSGGGGSDIQLTQSPSSLSASVGDRVSITCKASQDVSIAVAWYQQKPGKAPKLLIYSASYRYTGVPDRFSGSGSGTDFTLTISSLQPEDFAVYYCQQHYITPLTFGAGTKVDIKGGGGSGGGGSGGGGSQVQLQQSGSELKKPGASVKVSCKASGYTFTNYGMNWVKQAPGQGLKWMGWINTYTGEPTYTDDFKGRFAFSLDTSVSTAYLQISSLKADDTAVYFCARGGFGSSYWYFDVWGQGSLVTVSS

SEQ ID NO: 19 - protein, 214 aa, Artificial Sequence; identical to SEQ ID NO: 17
  Synthetic Construct

SEQ ID NO: 20 - protein, 701 aa, Artificial Sequence
  Synthetic Construct
QVQLQQSGSELKKPGASVKVSCKASGYTFTNYGMNWVKQAPGQGLKWMGWINTYTGEPTYTDDFKGRFAFSLDTSVSTAYLQISSLKADDTAVYFCARGGFGSSYWYFDVWGQGSLVTVSSASTKGPSVFPLAPSSKSTSGGTAALGCLVKDYFPEPVTVSWNSGALTSGVHTFPAVLQSSGLYSLSSVVTVPSSSLGTQTYICNVNHKPSNTKVDKRVEPKSCDKTHTCPPCPAPELLGGPSVFLFPPKPKDTLMISRTPEVTCVVVDVSHEDPEVKFNWYVDGVEVIINAKTKPREEQYNSTYRVVSVLTVLHQDWLNGKEYKCKVSNKALPAPIEKTISKAKGQPREPQVYTLPPSREEMTKNQVSLTCLVKGFYPSDIAVEWESNGQPENWKTTPPVLDSDGSFFLYSKLTVDKSRWQQGNVFSCSVMHEALHNHYTQKSLSLSPGGGGGSGGGGSDIQMTQSPSSISASVGDRVTTTCRASQDVNTAVAWYQQKPGKAPKLLIYSASFLYSGVPSRFSGSRSGTDFTLTISSLQPEDFATYYCQQHYTTPPTFGQGTKVEIKGGGGSGGGGSGGGGSEVQLVESGGGLVQPGGSLRLSCAASGFNIKDTYIHWVRQAPGKGLEWVARIYPTNGYTRYADSVKGRFTISADTSKNTAYLQNSLRAEDTAVYYCSRWGGDGFYAMDYWGQGTLVTVSS

SEQ ID NO: 21 - protein, 215 aa, Artificial Sequence
  Synthetic Construct
DIQLTQSPSSLSASVGDRVSITCKASQDVSIAVAWYQQKPGKAPKLLIYSASYRYTGVPDRFSGSGSGTDFTLTISSLQPEDFAVYYCQQHYITPLTFGAGTKVDIKRTVAAPSVFIFPPSDEQLKSGTASVVCLLNNFYPREAKVQWKVDNALQSGNSQESVTEQDSKDSTYSLSSTLTLSKADYEKHKVYACEVTIIQGLSSPVTKSFNRGEC

SEQ ID NO: 22 - protein, 703 aa, Artificial Sequence
  Synthetic Construct
DIQMTQSPSSLSASVGDRVTITCRASQDVNTAVAWYQQKPGKAPKLLIYSASFLYSGVPSRFSGSRSGTDFTLTISSLQPEDFATYYCQQHYTTPPTFGQGTKVEIKGGGGSGGGGSGGGGSEVQLVESGGGLVQPGGSLRLSCMSGFNIKDTYIHWVRQAPGKGLEWVARIYPTNGYTRYADSVKGRFTISADTSKNTAYLQMNSLRAEDTAVYYCSRWGGDGFYAMDYWGQGTLVTVSSGGGGSGGGGSGGGSQVQLQQSGSELKKPGASVKVSCKASGYTFTNYGMNWVKQAPGQGLWMGWINTYTGEPTYTDDFKGRFAFSLDTSVSTAYLQISSLKADDTAVYFCARGGFGSSYWYFDVWGQGSLVTVSSASTKGPSVFPLAPSSKSTSGGTAALGCLVKDYFPEPVTVSWNSGALTSGVHTFPAVLQSSGLYSLSSVVTVPSSSLGTQTYICWNHKPSNTKVDKRVEPKSCDKTHTCPPCPAPELLGGPSVFLFPPKPKDTLMISRTPEVTCVVVDVSHEDPEVKFNWYVDGVEVHNAKTKPREEQYNSTYRVVSVLTVLHQDWLNGKEYKCKVSNKALPAPTEKTTSKAKGQPREPQVYTLPPSREEMTKNQVSLTCLVKGFYPSDIAVEWESNGQPENNYKTTPPVLDSDGSFFLYSKLTVDKSRWQQGNVFSCSVMHEALRNHYTQKSLSLSPG

SEQ ID NO: 23 - protein, 215 aa, Artificial Sequence; identical to SEQ ID NO: 21
  Synthetic Construct

SEQ ID NO: 24 - protein, 10 aa, Artificial Sequence
  Synthetic Construct
GGGGSGGGGS

SEQ ID NO: 25 - protein, 14 aa, Artificial Sequence
  Synthetic Construct
GGGGSGGGGSGGGS

SEQ ID NO: 26 - protein, 5 aa, Artificial Sequence
  Synthetic Construct
SYGVN

SEQ ID NO: 27 - protein, 16 aa, Artificial Sequence
  Synthetic Construct
VMWAGGSTNYNSALMS

SEQ ID NO: 28 - protein, 11 aa, Artificial Sequence
  Synthetic Construct
DENWDGAWFAY

SEQ ID NO: 29 - protein, 17 aa, Artificial Sequence
  Synthetic Construct
KSSQSLLNSGTRKNYLA

SEQ ID NO: 30 - protein, 7 aa, Artificial Sequence
  Synthetic Construct
WASSRES

SEQ ID NO: 31 - protein, 8 aa, Artificial Sequence
  Synthetic Construct
KQSYNLFT

SEQ ID NO: 32 - protein, 5 aa, Artificial Sequence
  Synthetic Construct
DTYIH

SEQ ID NO: 33 - protein, 17 aa, Artificial Sequence
  Synthetic Construct
RIYPTNGYTRYADSVKG

SEQ ID NO: 34 - protein, 11 aa, Artificial Sequence
  Synthetic Construct
WGGDGFYAMDY

SEQ ID NO: 35 - protein, 11 aa, Artificial Sequence
  Synthetic Construct
RASQDVNTAVA

SEQ ID NO: 36 - protein, 7 aa, Artificial Sequence
  Synthetic Construct
SASFLYS

SEQ ID NO: 37 - protein, 9 aa, Artificial Sequence
  Synthetic Construct
QQHYTTPPT

SEQ ID NO: 38 - protein, 5 aa, Artificial Sequence
  Synthetic Construct
NYGMN

SEQ ID NO: 39 - protein, 17 aa, Artificial Sequence
  Synthetic Construct
WINTYTGEPTYTDDFKG

SEQ ID NO: 40 - protein, 12 aa, Artificial Sequence
  Synthetic Construct
GGFGSSYWYFDV

SEQ ID NO: 41 - protein, 11 aa, Artificial Sequence
  Synthetic Construct
KASQDVSIAVA

SEQ ID NO: 42 - protein, 7 aa, Artificial Sequence
  Synthetic Construct
SASYRYT

SEQ ID NO: 43 - protein, 9 aa, Artificial Sequence
  Synthetic Construct
QQHYITPLT

SEQ ID NO: 44 - protein, 5 aa, Artificial Sequence
  Synthetic Construct
GGGGS

SEQ ID NO: 45 - protein, 10 aa, Artificial Sequence
  Synthetic Construct
GGGGSGGGGS

SEQ ID NO: 46 - protein, 15 aa, Artificial Sequence
  Synthetic Construct
GGGGSGGGGSGGGGS

SEQ ID NO: 47 - protein, 20 aa, Artificial Sequence
  Synthetic Construct
GGGGSGGGGSGGGGSGGGGS

SEQ ID NO: 48 - protein, 1 aa, Artificial Sequence
  Synthetic Construct
  VARIANT 1: Can be present in repeats of any integer
G

SEQ ID NO: 49 - protein, 2 aa, Artificial Sequence
  Synthetic Construct
  VARIANT (1)..(2): Can be present in repeats of any integer up to and including 8
GS

SEQ ID NO: 50 - protein, 5 aa, Artificial Sequence
  Synthetic Construct
  VARIANT (1)..(5): Can be present in repeats of any integer up to and including 8
GSGGS

SEQ ID NO: 51 - protein, 5 aa, Artificial Sequence
  Synthetic Construct
  VARIANT (1)..(5): Can be present in repeats of any integer up to and including 8
GGGGS

SEQ ID NO: 52 - protein, 4 aa, Artificial Sequence
  Synthetic Construct
  VARIANT (1)..(4): Can be present in repeats of any integer up to and including 8
GGGS

SEQ ID NO: 53 - protein, 30 aa, Artificial Sequence
  Synthetic Construct
GGGGSGGGGSGGGGSGGGGSGGGGSGGGGS

SEQ ID NO: 54 - protein, 15 aa, Artificial Sequence
  Synthetic Construct
  VARIANT (1)..(15): Can be present in repeats of any integer up to and including 3
GSTSGSGKPGSGEGS

SEQ ID NO: 55 - protein, 119 aa, Artificial Sequence
  Synthetic Construct
EVQLVESGGGLVQPGGSLRLSCAASGFNIKDTYIHWVRQAPGKGLEWVARIYPTNGYTRYADSVKGRFTISADTSKNTAYLQNSLRAEDTAVYYCSRWGGDGFYAMDYWGQGTLVTVSS

SEQ ID NO: 56 - protein, 119 aa, Artificial Sequence
  Synthetic Construct
EVQLVESGGGLVQPGGSLRLSCMSGFNIKDTYIHWVRQAPGKGLEWVARIYPTNGYTRYADSVKGRFTISADTSKNTAYLQMNSLRAEDTAVYYCSRWGGDGFYAMDYWGQGTLVTVSS

SEQ ID NO: 57 - protein, 107 aa, Artificial Sequence
  Synthetic Construct
DIQMTQSPSSISASVGDRVTTTCRASQDVNTAVAWYQQKPGKAPKLLIYSASFLYSGVPSRFSGSRSGTDFTLTISSLQPEDFATYYCQQHYTTPPTFGQGTKVEIK

SEQ ID NO: 58 - protein, 120 aa, Artificial Sequence
  Synthetic Construct
QVQLQQSGSELKKPGASVKVSCKASGYTFTNYGMNWVKQAPGQGLWMGWINTYTGEPTYTDDFKGRFAFSLDTSVSTAYLQISSLKADDTAVYFCARGGFGSSYWYFDVWGQGSLVTVSS

SEQ ID NO: 59 - protein, 726 aa, Artificial Sequence
  Synthetic Construct
DIVMTQSPDSLAVSLGERATINCKSSQSLLNSGTRKNYLAWYQQKPGQPPKLLISWASSRESGVPDRFSGSGSGTDFTLTISSLQAEDVAVYYCKQSYNLFTFGGGTKVEIKGGGGSGGGGSGGGGSQVQLQESGPGLVKPSETLSLTCTVSGFSLTSYGVNWIRQPPGKGLEWIGVMWAGGSTNYNSALMSRLTISKDTSKNQFSLKLSSVTAADTAVYYCARDENWDGAWFAYWGQGTLVTVSSGGGGSGGGGSGGGGSGGGGSGGGGSGGGGSEVQLVESGGGLVQPGGSLRLSCAASGFNIKDTYIHWVRQAPGKGLEWVARIYPTNGYTRYADSVKGRFTISADTSKNTAYLQMNSLRAEDTAVYYCSRWGGDGFYAMDYWGQGTLVTVSSASTKGPSVFPLAPSSKSTSGGTAALGCLVKDYFPEPVTVSWNSGALTSGVHTFPAVLQSSGLYSLSSVVTVPSSSLGTQTYICNVNHKPSNTKVDKRVEPKSCDKTHTCPPCPAPELLGGPSVFLFPPKPKDTLMISRTPEVTCVVVDVSHEDPEVKFNWYVDGVEVHNAKTKPREEQYNSTYRVVSVLTVLHQDWLNGKEYKCKVSNKALPAPIEKTISKAKGQPREPQVYTLPPSREEMTKNQVSLTCLVKGFYPSDIAVEWESNGQPENNYKTTPPVLDSDGSFFLYSKLTVDKSRWQQGNVFSCSVMHEALHNHYTQKSLSLSPGK

SEQ ID NO: 60 - protein, 721 aa, Artificial Sequence
  Synthetic Construct
DIQMTQSPSSLSASVGDRVTITCRASQDVNTAVAWYQQKPGKAPKLLIYSASFLYSGVPSRFSGSRSGTDFTLTISSLQPEDFATYYCQQHYTTPPTFGQGTKVEIKGGGGSGGGGSGGGGSEVQLVESGGGLVQPGGSLRLSCAASGFNIKDTYIHWVRQAPGKGLEWVARIYPTNGYTRYADSVKGRFTISADTSKNTAYLQMNSLRAEDTAVYYCSRWGGDGFYAMDYWGQGTLVTVSSGGGGSGGGGSGGGGSGGGGSGGGGSGGGGSQVQLQESGPGLVKPSETLSLTCTVSGFSLTSYGVNWIRQPPGKGLEWIGVMWAGGSTNYNSALMSRLTISKDTSKNQFSLKLSSVTAADTAVYYCARDENWDGAWFAYWGQGTLVTVSSASTKGPSVFPLAPSSKSTSGGTAALGCLVKDYFPEPVTVSWNSGALTSGVHTFPAVLQSSGLYSLSSVVTVPSSSLGTQTYICNVNHKPSNTKVDKRVEPKSCDKTHTCPPCPAPELLGGPSVFLFPPKPKDTLMISRTPEVTCVVVDVSHEDPEVKFNWYVDGVEVHNAKTKPREEQYNSTYRVVSVLTVLHQDWLNGKEYKCKVSNKALPAPIEKTISKAKGQPREPQVYTLPPSREEMTKNQVSLTCLVKGFYPSDIAVEWESNGQPENNYKTTPPVLDSDGSFFLYSKLTVDKSRWQQGNVFSCSVMHEALHNHYTQKSLSLSPGK

SEQ ID NO: 61 - protein, 741 aa, Artificial Sequence
  Synthetic Construct
DIVMTQSPDSLAVSLGERATINCKSSQSLLNSGTRKNYLAWYQQKPGQPPKLLISWASSRESGVPDRFSGSGSGTDFTLTISSLQAEDVAVYYCKQSYNLFTFGGGTKVEIKGGGGSGGGGSGGGGSGGGGSGGGGSGGGGSQVQLQESGPGLVKPSETLSLTCTVSGFSLTSYGVNWIRQPPGKGLEWIGVMWAGGSTNYNSALMSRLTISKDTSKNQFSLKLSSVTAADTAVYYCARDENWDGAWFAYWGQGTLVTVSSGGGGSGGGGSGGGGSGGGGSGGGGSGGGGSEVQLVESGGGLVQPGGSLRLSCAASGFNIKDTYIHWVRQAPGKGLEWVARIYPTNGYTRYADSVKGRFTISADTSKNTAYLQMNSLRAEDTAVYYCSRWGGDGFYAMDYWGQGTLVTVSSASTKGPSVFPLAPSSKSTSGGTAALGCLVKDYFPEPVTVSWNSGALTSGVHTFPAVLQSSGLYSLSSVVTVPSSSLGTQTYICNVNHKPSNTKVDKRVEPKSCDKTHTCPPCPAPELLGGPSVFLFPPKPKDTLMISRTPEVTCVVVDVSHEDPEVKFNWYVDGVEVHNAKTKPREEQYNSTYRVVSVLTVLHQDWLNGKEYKCKVSNKALPAPIEKTISKAKGQPREPQVYTLPPSREEMTKNQVSLTCLVKGFYPSDIAVEWESNGQPENNYKTTPPVLDSDGSFFLYSKLTVDKSRWQQGNVFSCSVMHEALHNHYTQKSLSLSPGK

SEQ ID NO: 62 - protein, 736 aa, Artificial Sequence
  Synthetic Construct
DIQMTQSPSSLSASVGDRVTITCRASQDVNTAVAWYQQKPGKAPKLLIYSASFLYSGVPSRFSGSRSGTDFTLTISSLQPEDFATYYCQQHYTTPPTFGQGTKVEIKGGGGSGGGGSGGGGSGGGGSGGGGSGGGGSEVQLVESGGGLVQPGGSLRLSCAASGFNIKDTYIHWVRQAPGKGLEWVARIYPTNGYTRYADSVKGRFTISADTSKNTAYLQMNSLRAEDTAVYYCSRWGGDGFYAMDYWGQGTLVTVSSGGGGSGGGGSGGGGSGGGGSGGGGSGGGGSQVQLQESGPGLVKPSETLSLTCTVSGFSLTSYGVNWIRQPPGKGLEWIGVMWAGGSTNYNSALMSRLTISKDTSKNQFSLKLSSVTAADTAVYYCARDENWDGAWFAYWGQGTLVTVSSASTKGPSVFPLAPSSKSTSGGTAALGCLVKDYFPEPVTVSWNSGALTSGVHTFPAVLQSSGLYSLSSVVTVPSSSLGTQTYICNVNHKPSNTKVDKRVEPKSCDKTHTCPPCPAPELLGGPSVFLFPPKPKDTLMISRTPEVTCVVVDVSHEDPEVKFNWYVDGVEVHNAKTKPREEQYNSTYRVVSVLTVLHQDWLNGKEYKCKVSNKALPAPIEKTISKAKGQPREPQVYTLPPSREEMTKNQVSLTCLVKGFYPSDIAVEWESNGQPENNYKTTPPVLDSDGSFFLYSKLTVDKSRWQQGNVFSCSVMHEALHNHYTQKSLSLSPGK

SEQ ID NO: 63 - DNA, 12 bp, Artificial Sequence
  Synthetic Construct
aaatttcccggg